European Patent Application EP 4 414 377 A1, published August 14, 2024. Title: METHOD FOR OPTIMIZING VIRUS MEMBRANE FUSION INHIBITOR, BROAD-SPECTRUM ANTI-CORONA VIRUS LIPOPEPTIDE AND USE THEREOF. Applicant: Youcare Pharmaceutical Group Co., Ltd. The sequence listing filed with the application follows.

SEQUENCE LISTING (6 sequences)

SEQ ID NO: 1 - protein, 43 aa, Artificial Sequence
  synthetic peptide
SVVNIQKEIDRLNEVAKNLNESLIDLQELGKYEQYIKEAAAKK

SEQ ID NO: 2 - protein, 43 aa, Artificial Sequence
  synthetic peptide
SVVNIQKEIDRLNEVAKNLNESLIDLQELGKYEQYIKGSGSGK

SEQ ID NO: 3 - protein, 37 aa, Artificial Sequence
  synthetic peptide
SVVNIQKEIDRLNEVAKNLNESLIDLQELGKYEQYIK

SEQ ID NO: 4 - protein, 5 aa, Artificial Sequence
  synthetic peptide
EAAAK

SEQ ID NO: 5 - protein, 5 aa, Artificial Sequence
  synthetic peptide
GSGSG

SEQ ID NO: 6 - protein, 52 aa, Artificial Sequence
  synthetic peptide
FNGIGVTQNVLYENQKLIANQFNSAIGKIQDSLSSTASALGKLQDVVNQNAQ